European Patent Specification EP 3 469 078 B1, published March 27, 2024. Title: METHODS AND COMPOSITIONS FOR NUCLEIC ACID AMPLIFICATION. Applicant: LIFE TECHNOLOGIES CORPORATION YU, Hua NIKIFOROV, Theo ROSENBAUM, Abraham. Application To Be Assigned. The sequence listing filed with the application follows.

SEQUENCE LISTING (29 sequences)

SEQ ID NO: 1 - DNA, 202 bp, Artificial Sequence
  Synthetic DNA
acacggtccagactcctacgggaggcagcagtggggaatattgcacaatgggcgcaagcctgatgcagccatgccgcgtgtatgaagaaggccttcgggttgtaaagtactttcagcggggaggaagggagtaaagttaatacctttgctcattgacgttacccgcagaagaagcaccggctaactccgtgccagcagccgc

SEQ ID NO: 2 - DNA, 30 bp, Artificial Sequence
  Synthetic DNA
acacggtccadactcctacgggaggcagca

SEQ ID NO: 3 - DNA, 30 bp, Artificial Sequence
  Synthetic DNA
gcggctgctggcacggagttagccggtgct

SEQ ID NO: 4 - DNA, 47 bp, Artificial Sequence
  Synthetic DNA
acacggtccadactcctacgggaggcagcargtggggaatattgcac

SEQ ID NO: 5 - DNA, 47 bp, Artificial Sequence
  Synthetic DNA
gcggctgctggcacggagttagccggtgctructtctgcgggtaacg

SEQ ID NO: 6 - DNA, 50 bp, Artificial Sequence
  Synthetic DNA
cctatcccctgtgtgccttggcagtctcagccructctatgggcagtcga

SEQ ID NO: 7 - DNA, 34 bp, Artificial Sequence
  Synthetic DNA
ccactacgcctccgcttrucctctctatgggcag

SEQ ID NO: 8 - DNA, 34 bp, Artificial Sequence
  Synthetic DNA
cctccgctttcctctctratgggcagtcggtgat

SEQ ID NO: 9 - DNA, 20 bp, Artificial Sequence
  Synthetic DNA
ccatctcatccctgcgtgtc

SEQ ID NO: 10 - DNA, 26 bp, Artificial Sequence
  Synthetic DNA
ccatctcatccctgcgtgtctccgac

SEQ ID NO: 11 - DNA, 31 bp, Artificial Sequence
  Synthetic DNA
ccatctcatccctgcrgtgtctccgactcag

SEQ ID NO: 12 - DNA, 37 bp, Artificial Sequence
  Synthetic DNA
aacgatccatctcatccctgcrgtgtctccgactcag

SEQ ID NO: 13 - DNA, 20 bp, Artificial Sequence
  Synthetic DNA
ccatctcatccctgcgtgtc

SEQ ID NO: 14 - DNA, 57 bp, Artificial Sequence
  Synthetic DNA
gaatctgtccataaggtcagtaacgatccatctcatccctgcgtgtctccgactcag

SEQ ID NO: 15 - DNA, 53 bp, Artificial Sequence
  Synthetic DNA
cctatcccctgtgtgccttggcagtctcagcctctctatgggcagtcggtgat

SEQ ID NO: 16 - DNA, 31 bp, Artificial Sequence
  Synthetic DNA
ccatctcatccctgcgtgtctccgractcac

SEQ ID NO: 17 - DNA, 31 bp, Artificial Sequence
  Synthetic DNA
cctatcccctgtgtgccttggcargtctcac

SEQ ID NO: 18 - DNA, 49 bp, Artificial Sequence
  Synthetic DNA
gaatctgtccataaggtcagtaacgatccatrctcatccctgcgtgtca

SEQ ID NO: 19 - DNA, 54 bp, Artificial Sequence
  Synthetic DNA
cctatcccctgtgtgccttggcagtctcagcctctrctatgggcagtcggtgaa

SEQ ID NO: 20 - DNA, 48 bp, Artificial Sequence
  Synthetic DNA
gaatctgtccataaggtcagtaacgatccatrctcatccctgcgtgtc

SEQ ID NO: 21 - DNA, 52 bp, Artificial Sequence
  Synthetic DNA
cctatcccctgtgtgccttggcagtctcagcctctrctatgggcagtcggtg

SEQ ID NO: 22 - DNA, 47 bp, Artificial Sequence
  Synthetic DNA
gaatctgtccataaggtcagtaacgatccaructcatccctgcgtgt

SEQ ID NO: 23 - DNA, 38 bp, Artificial Sequence
  Synthetic DNA
gaatctgtccataaggtcagtaacgatccatrctcatc

SEQ ID NO: 24 - DNA, 42 bp, Artificial Sequence
  Synthetic DNA
cctatcccctgtgtgccttggcagtctcagcctctrctatgg

SEQ ID NO: 25 - DNA, 42 bp, Artificial Sequence
  Synthetic DNA
gaatctgtccataaggtcagtaacgatccaructcatccctg

SEQ ID NO: 26 - DNA, 32 bp, Artificial Sequence
  Synthetic DNA
gaatctgtccataagrgtcagtaacgatccat

SEQ ID NO: 27 - DNA, 34 bp, Artificial Sequence
  Synthetic DNA
cctatcccctgtgtgccrutggcagtctcagcct

SEQ ID NO: 28 - DNA, 46 bp, Artificial Sequence
  Synthetic DNA
gaatctgtccataaggtcagtaacgatccauctcatccctgcgtgt

SEQ ID NO: 29 - DNA, 48 bp, Artificial Sequence
  Synthetic DNA
cctatcccctgtgtgccttggcagtctcagccuctctatgggcagtcg